European Patent Specification EP 4 023 675 B1, published November 22, 2023. Title: Humanized antibody specific for CD22 and chimeric antigen receptor using the same. Applicant: InnoBation.Co., Ltd. The sequence listing filed with the application follows.

SEQUENCE LISTING (55 sequences)

SEQ ID NO: 1 - protein, 9 aa, Artificial
  2G1_VH_CDR1
GFSLTSYDI

SEQ ID NO: 2 - protein, 7 aa, Artificial
  2G1_VH_CDR2
IWTGGGT

SEQ ID NO: 3 - protein, 12 aa, Artificial
  2G1_VH_CDR3
VPHYYGYAMDYW

SEQ ID NO: 4 - protein, 6 aa, Artificial
  2G1_VL_CDR1
QDINKY

SEQ ID NO: 5 - protein, 3 aa, Artificial
  2G1_VL_CDR2
YTS

SEQ ID NO: 6 - protein, 8 aa, Artificial
  2G1_VL_CDR3
LQYDNLLT

SEQ ID NO: 7 - protein, 117 aa, Artificial
  2G1_VH
EVQLQESGPGLVAPSQSLSITCTVSGFSLTSYDISWIRQPPGKGLEWLGVIWTGGGTNYNSAFMSRLSISKDNSKSQVFLKMNSLQTDDTAIYYCVPHYYGYAMDYWGQGTSVTVSS

SEQ ID NO: 8 - protein, 106 aa, Artificial
  2G1_VL
DIVLTQSPSSLSASLGGKVTITCKASQDINKYIAWYQHKPGKGPRLLIHYTSTLQPGIPSRFSGSGSGRDYSFSISNLEPEDIATYYCLQYDNLLTFGAGTKLELK

SEQ ID NO: 9 - DNA, 351 bp, Artificial
  2G1_VH
gaggtgcagctgcaggagtcaggacctggcctggtggcgccctcacagagcctgtccattacctgcactgtctctgggttctcattaaccagctatgatataagctggattcgccagccaccaggaaagggtctggagtggcttggagtaatatggactggtggaggcacaaattataattcagctttcatgtccagactgagcatcagcaaggacaactccaagagccaagttttcttaaaaatgaacagtctgcaaactgatgacacagccatatattactgtgtccctcattactacggctatgctatggactactggggtcaaggaacctcagtcaccgtctcctca

SEQ ID NO: 10 - DNA, 318 bp, Artificial
  2G1_VL
gatattgtgctgacccagtctccatcctcactgtctgcatctctgggaggcaaagtcaccatcacttgcaaggcaagccaagacattaacaagtatatagcttggtaccaacacaagcctggaaaaggtcctaggctgctcatacattacacatctacattacagccaggcatcccatcaaggttcagtggaagtgggtctgggagagattattccttcagcatcagcaacctggagcctgaagatattgcaacttattattgtctacagtatgataatctgctcacgttcggtgctgggaccaagctggagctgaaa

SEQ ID NO: 11 - protein, 117 aa, Artificial
  2G1-V4_VH
EVQLQESGPGLVKPSQTLSLTCTVSGFSLTSYDISWIRQPPGKGLEWLGVIWTGGGTNYNSALKSRVTISKDNSKSQVSLKLSSVTAADTAVYYCVPHYYGYAMDYWGQGTTVTVSS

SEQ ID NO: 12 - protein, 106 aa, Artificial
  2G1-V4_VL
EIVLTQSPATLSLSPGERATLSCRASQDINKYIAWYQQKPGQAPRLLIHYTSTRQTGIPARFSGSGSGRDYTLTISSLEPEDFAVYYCLQYDNLLTFGGGTKLEIK

SEQ ID NO: 13 - DNA, 351 bp, Artificial
  2G1-V4_VH
gaggtgcagctgcaggagagcggccccggcctggtgaagccgagccagactctttctctgacctgcaccgtgtccggcttctctcttacgagctacgacatctcgtggatccggcagccgcctgggaaaggcttagagtggctaggggtgatttggaccggcgggggtaccaactacaactccgcgctcaaatcccgcgtcactatttctaaggacaattccaagagccaggtctcgctgaagctctcgtccgtgaccgccgcggacaccgcagtttattactgcgtgcctcattactacggctacgccatggattattggggccagggcaccacagtaacagtcagctcc

SEQ ID NO: 14 - DNA, 318 bp, Artificial
  2G1-V4_VL
gagatcgtgctgactcagagcccggccacccttagcctgagtccaggcgagcgcgctacgttgtcatgccgagcttcccaggacattaacaagtacatcgcgtggtaccagcagaagcccggacaggccccccgcctgctcatccactacacctccacccgccagactggcatccctgccaggttttcaggctccggttctggccgtgactacaccctgaccatctctagtttggagcccgaagatttcgccgtgtactactgtctgcaatatgacaacctgctgaccttcggagggggtaccaagctggagatcaag

SEQ ID NO: 15 - protein, 117 aa, Artificial
  2G1-V12_VH
EVQLKESGPVLVKPTETLTLTCTVSGFSLTSYDISWIRQPPGKALEWLGVIWTGGGTNYNSALKSRLTISKDNSKSQVVLTMTNMDPVDTATYYCVPHYYGYAMDYWGQGTTVTVSS

SEQ ID NO: 16 - protein, 106 aa, Artificial; identical to SEQ ID NO: 12
  2G1-V12_VL

SEQ ID NO: 17 - DNA, 351 bp, Artificial
  2G1-V12_VH
gaggtgcagctgaaggagagcgggccggtgctggtgaagcctaccgagactctgaccctgacctgcactgtttccggcttctctctgacgagctacgacatcagttggatccgccagccacccggcaaagcgttggaatggctcggggtaatttggaccggtggcgggaccaactacaacagcgcgctcaaatcgcggctaaccatctcaaaggacaactccaagtcccaagtggtgttaactatgacaaatatggatccggtcgacaccgctacctattactgcgtgcctcattactacggctacgccatggattattggggccagggcacgaccgtgaccgtctccagt

SEQ ID NO: 18 - DNA, 318 bp, Artificial
  2G1-V12_VL
gagatcgtgttgacccagagccctgccacgctgagcctgtcccccggggagcgcgccactctttcgtgtagggcttcccaggacattaacaagtacatcgcatggtaccagcagaagcccggacaggccccccgcctgctcatccactacacatccacccgccagacaggcatcccggctcgattctctggttctggcagcggtcgtgattacacccttactatttcttccctggagccagaggactttgcggtgtactactgcctgcagtatgacaacctgctgaccttcggcggaggcaccaagctggagatcaag

SEQ ID NO: 19 - protein, 15 aa, Artificial
  scfv linker
GGGGSGGGGSGGGGS

SEQ ID NO: 20 - DNA, 45 bp, Artificial
  scfv linker
ggcggaggcggcagcggcggaggcggctctggcggcggcgggagc

SEQ ID NO: 21 - DNA, 45 bp, Artificial
  scfv linker
gggggcggcggatctggtggtggaggctccggcggtggcggttcc

SEQ ID NO: 22 - DNA, 45 bp, Artificial
  scfv linker
ggcggcggtggctccggtggaggcggatctggcggtggcgggtcg

SEQ ID NO: 23 - protein, 238 aa, Artificial
  2G1 scfv
DIVLTQSPSSLSASLGGKVTITCKASQDINKYIAWYQHKPGKGPRLLIHYTSTLQPGIPSRFSGSGSGRDYSFSISNLEPEDIATYYCLQYDNLLTFGAGTKLELKGGGGSGGGGSGGGGSEVQLQESGPGLVAPSQSLSITCTVSGFSLTSYDISWIRQPPGKGLEWLGVIWTGGGTNYNSAFMSRLSISKDNSKSQVFLKMNSLQTDDTAIYYCVPHYYGYAMDYWGQGTSVTVSS

SEQ ID NO: 24 - DNA, 714 bp, Artificial
  2G1 scfv
gatatcgtgctgacccagagcccttctagcctgagcgcctctctgggcggcaaggtgaccatcacctgcaaggccagccaggacatcaacaagtacatcgcctggtaccagcacaagcctggaaaaggccctagactgctgatccactacaccagcacactccagcctggcatccccagcagattcagcggatctggaagcggcagagattacagcttcagcatttctaatctggaacctgaggacatcgctacatactattgtctgcagtacgacaacctgctgaccttcggcgctggcaccaagctggagctgaaaggcggaggcggcagcggcggaggcggctctggcggcggcgggagcgaggtgcagctgcaggagagcggccccggactggtcgccccaagccaatctctgtccatcacatgcaccgtgtccggctttagcctgacatcatatgatatcagctggatccggcagccacctggcaagggcctggaatggctgggcgttatctggaccggcggaggcacaaactacaactccgccttcatgagccggctgagcatctctaaggacaatagcaagtcccaggtgttcctgaagatgaacagcctgcaaacagacgacaccgccatctactactgcgtgccccactactacggctacgccatggactactggggccagggcaccagcgtgaccgtgtccagc

SEQ ID NO: 25 - protein, 238 aa, Artificial
  2G1-V4 scfv
EIVLTQSPATLSLSPGERATLSCRASQDINKYIAWYQQKPGQAPRLLIHYTSTRQTGIPARFSGSGSGRDYTLTISSLEPEDFAVYYCLQYDNLLTFGGGTKLEIKGGGGSGGGGSGGGGSEVQLQESGPGLVKPSQTLSLTCTVSGFSLTSYDISWIRQPPGKGLEWLGVIWTGGGTNYNSALKSRVTISKDNSKSQVSLKLSSVTAADTAVYYCVPHYYGYAMDYWGQGTTVTVSS

SEQ ID NO: 26 - DNA, 714 bp, Artificial
  2G1-V4 scfv
gagatcgtgctgactcagagcccggccacccttagcctgagtccaggcgagcgcgctacgttgtcatgccgagcttcccaggacattaacaagtacatcgcgtggtaccagcagaagcccggacaggccccccgcctgctcatccactacacctccacccgccagactggcatccctgccaggttttcaggctccggttctggccgtgactacaccctgaccatctctagtttggagcccgaagatttcgccgtgtactactgtctgcaatatgacaacctgctgaccttcggagggggtaccaagctggagatcaaggggggcggcggatctggtggtggaggctccggcggtggcggttccgaggtgcagctgcaggagagcggccccggcctggtgaagccgagccagactctttctctgacctgcaccgtgtccggcttctctcttacgagctacgacatctcgtggatccggcagccgcctgggaaaggcttagagtggctaggggtgatttggaccggcgggggtaccaactacaactccgcgctcaaatcccgcgtcactatttctaaggacaattccaagagccaggtctcgctgaagctctcgtccgtgaccgccgcggacaccgcagtttattactgcgtgcctcattactacggctacgccatggattattggggccagggcaccacagtaacagtcagctcc

SEQ ID NO: 27 - protein, 238 aa, Artificial
  2G1-V12 scfv
EIVLTQSPATLSLSPGERATLSCRASQDINKYIAWYQQKPGQAPRLLIHYTSTRQTGIPARFSGSGSGRDYTLTISSLEPEDFAVYYCLQYDNLLTFGGGTKLEIKGGGGSGGGGSGGGGSEVQLKESGPVLVKPTETLTLTCTVSGFSLTSYDISWIRQPPGKALEWLGVIWTGGGTNYNSALKSRLTISKDNSKSQVVLTMTNMDPVDTATYYCVPHYYGYAMDYWGQGTTVTVSS

SEQ ID NO: 28 - DNA, 714 bp, Artificial
  2G1-V12 scfv
gagatcgtgttgacccagagccctgccacgctgagcctgtcccccggggagcgcgccactctttcgtgtagggcttcccaggacattaacaagtacatcgcatggtaccagcagaagcccggacaggccccccgcctgctcatccactacacatccacccgccagacaggcatcccggctcgattctctggttctggcagcggtcgtgattacacccttactatttcttccctggagccagaggactttgcggtgtactactgcctgcagtatgacaacctgctgaccttcggcggaggcaccaagctggagatcaagggcggcggtggctccggtggaggcggatctggcggtggcgggtcggaggtgcagctgaaggagagcgggccggtgctggtgaagcctaccgagactctgaccctgacctgcactgtttccggcttctctctgacgagctacgacatcagttggatccgccagccacccggcaaagcgttggaatggctcggggtaatttggaccggtggcgggaccaactacaacagcgcgctcaaatcgcggctaaccatctcaaaggacaactccaagtcccaagtggtgttaactatgacaaatatggatccggtcgacaccgctacctattactgcgtgcctcattactacggctacgccatggattattggggccagggcacgaccgtgaccgtctccagt

SEQ ID NO: 29 - DNA, 1178 bp, Artificial
  EF1 promoter
gctccggtgcccgtcagtgggcagagcgcacatcgcccacagtccccgagaagttggggggaggggtcggcaattgaaccggtgcctagagaaggtggcgcggggtaaactgggaaagtgatgtcgtgtactggctccgcctttttcccgagggtgggggagaaccgtatataagtgcagtagtcgccgtgaacgttctttttcgcaacgggtttgccgccagaacacaggtaagtgccgtgtgtggttcccgcgggcctggcctctttacgggttatggcccttgcgtgccttgaattacttccacctggctgcagtacgtgattcttgatcccgagcttcgggttggaagtgggtgggagagttcgaggccttgcgcttaaggagccccttcgcctcgtgcttgagttgaggcctggcctgggcgctggggccgccgcgtgcgaatctggtggcaccttcgcgcctgtctcgctgctttcgataagtctctagccatttaaaatttttgatgacctgctgcgacgctttttttctggcaagatagtcttgtaaatgcgggccaagatctgcacactggtatttcggtttttggggccgcgggcggcgacggggcccgtgcgtcccagcgcacatgttcggcgaggcggggcctgcgagcgcggccaccgagaatcggacgggggtagtctcaagctggccggcctgctctggtgcctggcctcgcgccgccgtgtatcgccccgccctgggcggcaaggctggcccggtcggcaccagttgcgtgagcggaaagatggccgcttcccggccctgctgcagggagctcaaaatggaggacgcggcgctcgggagagcgggcgggtgagtcacccacacaaaggaaaagggcctttccgtcctcagccgtcgcttcatgtgactccactgagtaccgggcgccgtccaggcacctcgattagttctcgagcttttggagtacgtcgtctttaggttggggggaggggttttatgcgatggagtttccccacactgagtgggtggagactgaagttaggccagcttggcacttgatgtaattctccttggaatttgccctttttgagtttggatcttggttcattctcaagcctcagacagtggttcaaagtttttttcttccatttcaggtgtcgtga

SEQ ID NO: 30 - DNA, 63 bp, Artificial
  signal peptide
atggccttaccagtgaccgccttgctcctgccgctggccttgctgctccacgccgccaggccg

SEQ ID NO: 31 - DNA, 135 bp, Artificial
  CD8 Hinge
accacgacgccagcgccgcgaccaccaacaccggcgcccaccatcgcgtcgcagcccctgtccctgcgcccagaggcgtgccggccagcggcggggggcgcagtgcacacgagggggctggacttcgcctgtgat

SEQ ID NO: 32 - DNA, 72 bp, Artificial
  transmembrane domain
atctacatctgggcgcccttggccgggacttgtggggtccttctcctgtcactggttatcaccctttactgc

SEQ ID NO: 33 - DNA, 126 bp, Artificial
  4-1BB
aaacggggcagaaagaaactcctgtatatattcaaacaaccatttatgagaccagtacaaactactcaagaggaagatggctgtagctgccgatttccagaagaagaagaaggaggatgtgaactg

SEQ ID NO: 34 - DNA, 336 bp, Artificial
  CD3 zeta
agagtgaagttcagcaggagcgcagacgcccccgcgtacaagcagggccagaaccagctctataacgagctcaatctaggacgaagagaggagtacgatgttttggacaagagacgtggccgggaccctgagatggggggaaagccgagaaggaagaaccctcaggaaggcctgtacaatgaactgcagaaagataagatggcggaggcctacagtgagattgggatgaaaggcgagcgccggaggggcaaggggcacgatggcctttaccagggtctcagtacagccaccaaggacacctacgacgcccttcacatgcaggccctgccccctcgc

SEQ ID NO: 35 - DNA, 591 bp, Artificial
  WPRE
atcaacctctggattacaaaatttgtgaaagattgactggtattcttaactatgttgctccttttacgctatgtggatacgctgctttaatgcctttgtatcatgctattgcttcccgtatggctttcattttctcctccttgtataaatcctggttgctgtctctttatgaggagttgtggcccgttgtcaggcaacgtggcgtggtgtgcactgtgtttgctgacgcaacccccactggttggggcattgccaccacctgtcagctcctttccgggactttcgctttccccctccctattgccacggcggaactcatcgccgcctgccttgcccgctgctggacaggggctcggctgttgggcactgacaattccgtggtgttgtcggggaagctgacgtcctttccatggctgctcgcctgtgttgccacctggattctgcgcgggacgtccttctgctacgtcccttcggccctcaatccagcggaccttccttcccgcggcctgctgccggctctgcggcctcttccgcgtcttcgccttcgccctcagacgagtcggatctccctttgggccgcctccccgcctg

SEQ ID NO: 36 - protein, 21 aa, Artificial
  signal peptide
MALPVTALLLPLALLLHAARP

SEQ ID NO: 37 - protein, 45 aa, Artificial
  CD8 Hinge
TTTPAPRPPTPAPTIASQPLSLRPEACRPAAGGAVHTRGLDFACD

SEQ ID NO: 38 - protein, 24 aa, Artificial
  transmembrane domain
IYIWAPLAGTCGVLLLSLVITLYC

SEQ ID NO: 39 - protein, 42 aa, Artificial
  4-1BB
KRGRKKLLYIFKQPFMRPVQTTQEEDGCSCRFPEEEEGGCEL

SEQ ID NO: 40 - protein, 112 aa, Artificial
  CD3 zeta
RVKFSRSADAPAYKQGQNQLYNELNLGRREEYDVLDKRRGRDPEMGGKPRRKNPQEGLYNELQKDKMAEAYSEIGMKGERRRGKGHDGLYQGLSTATKDTYDALHMQALPPR

SEQ ID NO: 41 - protein, 8 aa, Artificial
  CD19_VH_CDR1
GVSLPDYG

SEQ ID NO: 42 - protein, 7 aa, Artificial
  CD19_VH_CDR2
IWGSETT

SEQ ID NO: 43 - protein, 14 aa, Artificial
  CD19_VH_CDR3
AKHYYYGGSYAMDY

SEQ ID NO: 44 - protein, 6 aa, Artificial
  CD19_VL_CDR1
QDISKY

SEQ ID NO: 45 - protein, 3 aa, Artificial
  CD19_VL_CDR2
HTS

SEQ ID NO: 46 - protein, 9 aa, Artificial
  CD19_VL_CDR3
QQGNTLPYT

SEQ ID NO: 47 - protein, 119 aa, Artificial
  CD19_VH
EVKLQESGPGLVAPSQSLSVTCTVSGVSLPDYGVSWIRQPPRKGLEWLGVIWGSETTYYNSALKSRLTIIKDNSKSQVFLKMNSLQTDDTAIYYCAKHYYYGGSYAMDYWGQGTSVTVS

SEQ ID NO: 48 - protein, 128 aa, Artificial
  CD19_VL
MALPVTALLLPLALLLHAARPDIQMTQTTSSLSASLGDRVTISCRASQDISKYLNWYQQKPDGTVKLLIYHTSRLHSGVPSRFSGSGSGTDYSLTISNLEQEDIATYFCQQGNTLPYTFGGGTKLEIT

SEQ ID NO: 49 - DNA, 360 bp, Artificial
  CD19_VH
tctgaggtgaaactgcaggagtcaggacctggcctggtggcgccctcacagagcctgtccgtcacatgcactgtctcaggggtctcattacccgactatggtgtaagctggattcgccagcctccacgaaagggtctggagtggctgggagtaatatggggtagtgaaaccacatactataattcagctctcaaatccagactgaccatcatcaaggacaactccaagagccaagttttcttaaaaatgaacagtctgcaaactgatgacacagccatttactactgtgccaaacattattactacggtggtagctatgctatggactactggggccaaggaacctcagtcaccgtctcc

SEQ ID NO: 50 - DNA, 384 bp, Artificial
  CD19_VL
atggccttaccagtgaccgccttgctcctgccgctggccttgctgctccacgccgccaggccggacatccagatgacacagactacatcctccctgtctgcctctctgggagacagagtcaccatcagttgcagggcaagtcaggacattagtaaatatttaaattggtatcagcagaaaccagatggaactgttaaactcctgatctaccatacatcaagattacactcaggagtcccatcaaggttcagtggcagtgggtctggaacagattattctctcaccattagcaacctggagcaagaagatattgccacttacttttgccaacagggtaatacgcttccgtacacgttcggaggggggaccaagctggagatcaca

SEQ ID NO: 51 - protein, 5 aa, Artificial
  Bi-specific CART linker
GGGGS

SEQ ID NO: 52 - DNA, 15 bp, Artificial
  Bi-specific CART linker
ggcgggggaggctct

SEQ ID NO: 53 - DNA, 15 bp, Artificial
  Bi-specific CART linker
ggcggagggggctcc

SEQ ID NO: 54 - protein, 18 aa, Artificial
  Bi-specific CART linker
GSTSGSGKPGSGEGSTKG

SEQ ID NO: 55 - DNA, 54 bp, Artificial
  Bi-specific CART linker
ggctccaccagtggttctgggaaacctggtagtggggagggctcgacgaagggg